European Patent Specification EP 3 497 449 B1, published August 21, 2024. Title: DETERMINATION OF NON-HUMAN MAMMAL TK1 PROTEIN LEVELS. Applicant: ALERTIX VETERINARY DIAGNOSTICS AB. The sequence listing filed with the application follows.

SEQUENCE LISTING (18 sequences)

SEQ ID NO: 1 - protein, 16 aa, Canis lupus
GKPGEGKEATGVRKLF

SEQ ID NO: 2 - protein, 23 aa, Homo sapiens
  ref <302>: Exposed proliferation-related peptides, ligands and methods employing the same
  ref <310>: WO 2008/142664
  ref <311>: 2008-05-23
  ref <312>: 2008-11-27
  ref <313>: (1)..(23)
AYTKRLGTEKEVEVIGGADKYHS

SEQ ID NO: 3 - protein, 242 aa, Canis lupus
MSCINLPTVLPGSPSKTRGQIQVILGPMFSGKSTELMRRVRRFQIAQYKCLVIKYAKDTRYSNSFSTHDRNTMEALPACLLRDVAQEALGVAVIGIDEGQFFPDIVEFSETMANAGKTVIVAALDGTFQRKAFGTILNLVPLAESVVKLTAVCMECFREAAYTKRLGSEKEVEVIGGADKYHSVCRLCYFKKASGPPMGLDSRENKENVLVLVPGKPGEGKEATGVRKLFAPQHVLQCSPAN

SEQ ID NO: 4 - protein, 234 aa, Homo sapiens
MSCINLPTVLPGSPSKTRGQIQVILGPMFSGKSTELMRRVRRFQIAQYKCLVIKYAKDTRYSSSFCTHDRNTMEALPACLLRDVAQEALGVAVIGIDEGQFFPDIVEFCEAMANAGKTVIVAALDGTFQRKPFGAILNLVPLAESVVKLTAVCMECFREAAYTKRLGTEKEVEVIGGADKYHSVCRLCYFKKASGQPAGPDNKENCPVPGKPGEAVAARKLFAPQQILQCSPAN

SEQ ID NO: 5 - protein, 17 aa, Canis lupus
CGKPGEGKEATGVRKLF

SEQ ID NO: 6 - protein, 24 aa, Homo sapiens
CAYTKRLGTEKEVEVIGGADKYHS

SEQ ID NO: 7 - protein, 23 aa, Canis lupus
AYTKRLGSEKEVEVIGGADKYHS

SEQ ID NO: 8 - protein, 24 aa, Canis lupus
CAYTKRLGSEKEVEVIGGADKYHS

SEQ ID NO: 9 - protein, 237 aa, Felis catus
MSCINLPTVLPGSPSKTRGQIQVILGPMFSGKSTELMRRVRRFQIAQYKCLVIKYAKDTRYSSSFSTHDRNTMEALPACLLRDVAQEALGVAVIGIDEGQFFPDIVEYSETMANAGKTVIVAALDGTFQRKAFGTILNLVPLAESVVKLTAVCMECFREAAYTKRLGAEKEVEVIGGADKYHSVCRLCYFKKASGLPAGPDGKENKENCPLLGKPGEASGARKLFAPHQILQCSSAN

SEQ ID NO: 10 - protein, 237 aa, Equus caballus
MSCINLPTVLPGSPSKTRGQIQVILGPMFSGKSTELMRRVRRFQIAQYKCLVIKYAKDTRYSSNFSTHDRNTMEALPACQLRDAAQEALGVAVIGIDEGQFFPDIVEFSEAMANAGKTVIVAALDGTFQRKAFGAILNLVPLAESVVKLTAVCMECFREAAYTKRLGTEKEVEVIGGADKYHSVCRLCYFKKPLGQPAGLDSTENKENFPVLGKPGEATGARKLFAPHQILQCSTAN

SEQ ID NO: 11 - protein, 15 aa, Canis lupus
VLVPGKPGEGKEATG

SEQ ID NO: 12 - protein, 16 aa, Canis lupus
CVLVPGKPGEGKEATG

SEQ ID NO: 13 - protein, 15 aa, Felis catus
GKPGEASGARKLFAP

SEQ ID NO: 14 - protein, 16 aa, Felis catus
CGKPGEASGARKLFAP

SEQ ID NO: 15 - protein, 23 aa, Felis catus
AYTKRLGAEKEVEVIGGADKYHS

SEQ ID NO: 16 - protein, 24 aa, Felis catus
CAYTKRLGAEKEVEVIGGADKYHS

SEQ ID NO: 17 - protein, 210 aa, Equus caballus
MFSGKSTELMRRVRRFQIAQYKCLVIKYAKDTRYSSNFSTHDRNTMEALPACQLRDAAQEALGVAVIGIDEGQFFPDIVEFSEAMANAGKTVIVAALDGTFQRKAFGAILNLVPLAESVVKLTAVCMECFREAAYTKRLGTEKEVEVIGGADKYHSVCRLCYFKKPLGQPAGLDSTENKENFPVLGKPGEATGARKLFAPHQILQCSTAN

SEQ ID NO: 18 - protein, 27 aa, Canis lupus
MSCINLPTVLPGSPSKTRGQIQVILGP